European Patent Application EP 4 509 180 A2, published February 19, 2025. Title: HUMANIZED ANTI-CLAUDIN-1 ANTIBODIES AND USES THEREOF. Applicant: INSERM (Institut National de la Santé et de la Recherche Médicale). Application EP Divisional of EP17710993.1, filed March 21, 2017. The sequence listing filed with the application follows.

SEQUENCE LISTING (12 sequences)

SEQ ID NO: 1 - protein, 119 aa, synthetic construct
  REGION 1..119: note = Humanized H3
QVQLVESGGGVVQPGRSLRLSCLGSGFSFSSYGMNWVRQAPGKGLEWVASISPSGSYFYYADSVKGRFTISRDNSKNTLYLQMTSLRAEDTAIYYCARLPGFNPPFDHWGQGTLVTVSS

SEQ ID NO: 2 - protein, 107 aa, synthetic construct
  REGION 1..107: note = humanized L3
DIQMTQSPSSLSASVGDRVTITCKASQNVGGNVDWYQWKPGKAPKLLIYGASNRYTGVPDRFRGSGSGTDFTLTISSLQPEDVATYYCLQYKNNPWTFGGGTKVEIK

SEQ ID NO: 3 - protein, 119 aa, Rattus norvegicus
EVQLVESGGGLVQPGRSLKLSCLGSGFSFSSYGMNWIRQAPGKGLEWVASISPSGSYFYYADSVKGRFTISRENAKNTLYLQMTSLRAEDTALYYCARLPGFNPPFDHWGQGVVVTVSS

SEQ ID NO: 4 - protein, 107 aa, Rattus norvegicus
NTVMTQSPTSMFMSVGDRVTMNCKASQNVGGNVDWYQWKPGQSPKLLMYGASNRYTGVPDRFRGSGSGTDFTLTISNMQTEDLAVYYCLQYKNNPWTFGGGTKVELK

SEQ ID NO: 5 - protein, 113 aa, Rattus norvegicus
EVQLVESGGGLVQPGRSLKLSCVASGFTFSDYRMNWIRQAPGKGLEWVASISSSSSYIYYADTVKGFTISRDNAKDTLYLQMTSLRSEDTALYYCARDYFDYWGQGVMVTVSS

SEQ ID NO: 6 - protein, 107 aa, Rattus norvegicus
NTVMTQSPTSMFISVGDRVTMNCKASQNVGTNVDWYQQKTGQSPKLLIYGASNRYTGVPDRFTGSGSGTDFTLTISNMQAEDLAVYYCLQYNYNPWTFGGGTKLELK

SEQ ID NO: 7 - protein, 114 aa, Homo sapiens
EVQLVESGGGLVKPGGSLRLSCAASGFTFSSYSMNWVRQAPGKGLEWVSSISSSSSYIYYADSVKGRFTISRDNAKNSLYLQMNSLRAEDTAVYYCARDAFDVWGQGTMVTVSS

SEQ ID NO: 8 - protein, 107 aa, Homo sapiens
EIVMTQSPATLSVSPGERATLSCRASQSVSSNLAWYQQKPGQAPRLLIYGASTRATGIPARFSGSGSGTEFTLTISSLQSEDFAVYYCQQYNNWPWTFGQGTKVEIK

SEQ ID NO: 9 - protein, 119 aa, synthetic construct
  REGION 1..119: note = Humanized H1
EVQLVESGGGLVKPGGSLRLSCAASGFSFSSYGMNWVRQAPGKGLEWVSSISPSGSYFYYADSVKGRFTISRDNAKNSLYLQMNSLRAEDTAVYYCARLPGFNPPFDHWGQGTLVTVSS

SEQ ID NO: 10 - protein, 107 aa, synthetic construct
  REGION 1..107: note = humanized L1
DIQMTQSPATLSVSPGERATLSCKASQNVGGNVDWYQWKPGQAPRLLIYGASNRYTGIPARFRGSGSGTEFTLTISSLQSEDFAVYYCLQYKNNPWTFGQGTKVEIK

SEQ ID NO: 11 - protein, 119 aa, synthetic construct
  REGION 1..119: note = humanized H2
QVQLVESGGGVVQPGRSLRLSCAASGFSFSSYGMNWVRQAPGKGLEWVTSISPSGSYFYYADSVKGRFTISRDNSKNTLYLQMNSLRAEDTAIYYCARLPGFNPPFDHWGQGTLVTVSS

SEQ ID NO: 12 - protein, 107 aa, synthetic construct
  REGION 1..107: note = humanized L2
DIQMTQSPSSLSASVGDRVTITCKASQNVGGNVDWYQWKPGKAPKLLIYGASNRYTGVPSRFRGSGSGTDFTLTISSLQPEDVATYYCLQYKNNPWTFGQGTKVEIK